European Patent Specification EP 3 733 844 B1, published April 2, 2025. Title: Composition for Altering Target Gene. Applicant: KYOTO UNIVERSITY TAKEDA PHARMACEUTICAL COMPANY LIMITED. The sequence listing filed with the application follows.

SEQUENCE LISTING (22 sequences)

SEQ ID NO: 1 - RNA, 96 nt, Artificial Sequence
  HsDMDEx45#1 sgRNA
  modified_base (1)..(1): n stands for uracil (u) which may be 2'-O-methyluridine (um)
  misc_feature (1)..(3): n is a, c, g, or u
  modified_base (2)..(2): n stands for guanine (g) which may be 2'-O-methylguanosine (gm)
  modified_base (3)..(3): n stands for guanine (g) which may be 2'-O-methylguanosine (gm)
  modified_base (93)..(93): n stands for guanine (g) which may be 2'-O-methylguanosine (gm)
  misc_feature (93)..(95): n is a, c, g, or u
  modified_base (94)..(94): n stands for uracil (u) which may be 2'-O-methyluridine (um)
  modified_base (95)..(95): n stands for guanine (g) which may be 2'-O-methylguanosine (gm)
nnnuaucuuacaggaacuccguuuuagagcuagaaauagcaaguuaaaauaaggcuaguccguuaucaacuugaaaaaguggcaccgagucgnnnc

SEQ ID NO: 2 - RNA, 96 nt, Artificial Sequence
  HsDmdEx45#23 sgRNA
  modified_base (1)..(1): n stands for adenine (a) which may be 2'-O-methyladenosine
  misc_feature (1)..(3): n is a, c, g, or u
  modified_base (2)..(2): n stands for guanine (g) which may be 2'-O-methylguanosine (gm)
  modified_base (3)..(3): n stands for cytosine (c) which may be 2'-O-methylcytidine (cm)
  modified_base (93)..(93): n stands for guanine (g) which may be 2'-O-methylguanosine (gm)
  misc_feature (93)..(95): n is a, c, g, or u
  modified_base (94)..(94): n stands for uracil (u) which may be 2'-O-methyluridine (um)
  modified_base (95)..(95): n stands for guanine (g) which may be 2'-O-methylguanosine (gm)
nnnugucagacagaaaaaagguuuuagagcuagaaauagcaaguuaaaauaaggcuaguccguuaucaacuugaaaaaguggcaccgagucgnnnc

SEQ ID NO: 3 - RNA, 20 nt, Artificial Sequence
  Target-recognizing sequence of HsDmdEX#1 sgRNA
  modified_base (1)..(1): n stands for uracil (u) which may be 2'-O-methyluridine (um)
  misc_feature (1)..(3): n is a, c, g, or u
  modified_base (2)..(2): n stands for guanine (g) which may be 2'-O-methylguanosine (gm)
  modified_base (3)..(3): n stands for guanine (g) which may be 2'-O-methylguanosine (gm)
nnnuaucuuacaggaacucc

SEQ ID NO: 4 - RNA, 20 nt, Artificial Sequence
  Target-recognizing sequence of HsDmdEX#23 sgRNA
  modified_base (1)..(1): n stands for adenine (a) which may be 2'-O-methyladenosine
  misc_feature (1)..(3): n is a, c, g, or u
  modified_base (2)..(2): n stands for guanine (g) which may be 2'-O-methylguanosine (gm)
  modified_base (3)..(3): n stands for cytosine (c) which may be 2'-O-methylcytidine (cm)
nnnugucagacagaaaaaag

SEQ ID NO: 5 - RNA, 32 nt, Artificial Sequence
  crRNA sequence of HsDmdEX#1 sgRNA
  modified_base (1)..(1): n stands for uracil (u) which may be 2'-O-methyluridine (um)
  misc_feature (1)..(3): n is a, c, g, or u
  modified_base (2)..(2): n stands for guanine (g) which may be 2'-O-methylguanosine (gm)
  modified_base (3)..(3): n stands for guanine (g) which may be 2'-O-methylguanosine (gm)
nnnuaucuuacaggaacuccguuuuagagcua

SEQ ID NO: 6 - RNA, 32 nt, Artificial Sequence
  crRNA sequence of HsDmdEX#23 sgRNA
  modified_base (1)..(1): n stands for adenine (a) which may be 2'-O-methyladenosine
  misc_feature (1)..(3): n is a, c, g, or u
  modified_base (2)..(2): n stands for guanine (g) which may be 2'-O-methylguanosine (gm)
  modified_base (3)..(3): n stands for cytosine (c) which may be 2'-O-methylcytidine (cm)
nnnugucagacagaaaaaagguuuuagagcua

SEQ ID NO: 7 - RNA, 60 nt, Artificial Sequence
  tracrRNA sequence of HsDmdEX#1 sgRNA
  modified_base (57)..(57): n stands for guanine (g) which may be 2'-O-methylguanosine (gm)
  misc_feature (57)..(59): n is a, c, g, or u
  modified_base (58)..(58): n stands for uracil (u) which may be 2'-O-methyluridine (um)
  modified_base (59)..(59): n stands for guanine (g) which may be 2'-O-methylguanosine (gm)
uagcaaguuaaaauaaggcuaguccguuaucaacuugaaaaaguggcaccgagucgnnnc

SEQ ID NO: 8 - RNA, 60 nt, Artificial Sequence; identical to SEQ ID NO: 7
  tracrRNA sequence of HsDmdEX#23 sgRNA
  modified_base (57)..(57): n stands for guanine (g) which may be 2'-O-methylguanosine (gm)
  misc_feature (57)..(59): n is a, c, g, or u
  modified_base (58)..(58): n stands for uracil (u) which may be 2'-O-methyluridine (um)
  modified_base (59)..(59): n stands for guanine (g) which may be 2'-O-methylguanosine (gm)

SEQ ID NO: 9 - RNA, 98 nt, Artificial Sequence
  MmRosa26 sgRNA
  modified_base (1)..(1): gm
  misc_feature (1)..(3): n is a, c, g, or u
  modified_base (3)..(3): um
  modified_base (95)..(95): um
  misc_feature (95)..(97): n is a, c, g, or u
  modified_base (96)..(96): um
  modified_base (97)..(97): um
nnngggcgggagucuucuguuuuagagcuagaaauagcaaguuaaaauaaggcuaguccguuaucaacuugaaaaaguggcaccgagucggugcnnnu

SEQ ID NO: 10 - DNA, 35 bp, Artificial Sequence
  Forward primer used in Example 1[1-3]
ctccgaggcggatcacaagcaataataacctgtag

SEQ ID NO: 11 - DNA, 35 bp, Artificial Sequence
  Reverse primer used in Example 1[1-3]
tgcaagcacgtttccgacttgagttgcctcaagag

SEQ ID NO: 12 - DNA, 20 bp, Mus musculus
atgaatgtgcctacatatgg

SEQ ID NO: 13 - DNA, 20 bp, Mus musculus
catagcatgcatttggcttc

SEQ ID NO: 14 - DNA, 20 bp, Mus musculus
gaatgaggtagtgttgtagg

SEQ ID NO: 15 - DNA, 20 bp, Mus musculus
gcaggaaatcatcttatagc

SEQ ID NO: 16 - DNA, 120 bp, Artificial Sequence
  ssODN used in Example 2[2-3]
gagcaagctgggttagaacaaaggtctgtcagagtcagcatgggaatgaggtagtgttgtagcaggaaatagtgtggtttaggtctctccccgccctctgtgtatgtgtgtgtgtgtgtt

SEQ ID NO: 17 - DNA, 35 bp, Artificial Sequence
  Forward primer used in Example 2[2-4] and [2-5], and Example 5
caagtttaaaatagcagaaaaccactaactagcca

SEQ ID NO: 18 - DNA, 35 bp, Artificial Sequence
  Reverse primer used in Example 2[2-4] and [2-5], and Example 5
ctgacacataaaaggtgtctttctgtcttgtatcc

SEQ ID NO: 19 - DNA, 21 bp, Artificial Sequence
  Forward primer used in Example 2[2-5] and Example 6
ggtgaaagtacaggaagccgt

SEQ ID NO: 20 - DNA, 21 bp, Artificial Sequence
  Reverse primer used in Example 2[2-5] and Example 6
ttagctgctgctcatctccaa

SEQ ID NO: 21 - DNA, 20 bp, Artificial Sequence
  Forward primer used in Example 3[3-5] and Example 4[4-5]
ctacaggaagctctctccca

SEQ ID NO: 22 - DNA, 22 bp, Artificial Sequence
  Reverse primer used in Example 3[3-5] and Example 4[4-5]
tgcttcctccaaccataaaaca